European Patent Specification EP 3 585 395 B1, published July 1, 2026. Title: TREATMENT OF LOWER URINARY TRACT EPITHELIUM WITH GLUCAGON LIKE PEPTIDE 2. Applicant: URIGEN N.A. The sequence listing filed with the application follows.

SEQUENCE LISTING (63 sequences)

SEQ ID NO: 1 - protein, 33 aa, Homo sapiens
HADGSFSDEMNTILDNLAARDFINWLIQTKITD

SEQ ID NO: 2 - protein, 33 aa, Artificial Sequence
  Description of Artificial Sequence: Synthetic polypeptide
HGDGSFSDEMNTILDNLAARDFINWLIQTKITD

SEQ ID NO: 3 - protein, 37 aa, Artificial Sequence
  Description of Artificial Sequence: Synthetic polypeptide
  MOD_RES (1)..(1): Arg, Lys, His, or absent
  MOD_RES (2)..(2): Arg, Lys, His, or absent
  MOD_RES (3)..(3): His or Tyr
  MOD_RES (4)..(4): Ala or an Ala-replacement amino acid conferring on said analog resistance to DPP-IV enzyme
  MOD_RES (5)..(5): Asp or Glu
  MOD_RES (6)..(6): Gly or Ala
  MOD_RES (11)..(11): Glu or Tyr
  MOD_RES (12)..(12): Ser if position 11 is Tyr, otherwise Met or an oxidatively stable Met replacement amino acid
  MOD_RES (13)..(13): Lys if position 11 is Tyr, or Asn
  MOD_RES (14)..(14): Tyr if position 11 is Tyr, or Thr
  MOD_RES (15)..(15): Ile, or Xaa is not present if position 11 is Tyr
  MOD_RES (21)..(21): Ala or Thr
  MOD_RES (22)..(22): Arg, Lys, His, or Ala
  MOD_RES (25)..(25): Ile or Val
  MOD_RES (26)..(26): Asn or Ala if position 25 is Ile, Gln if position 25 is Val
  MOD_RES (33)..(33): Ile or a covalent bond
  MOD_RES (34)..(34): Thr if position 34 is Ile, or a covalent bond
  MOD_RES (35)..(35): Asp if position 35 is Thr, or a covalent bond
  MOD_RES (36)..(36): Arg, Lys, His, or absent
  MOD_RES (37)..(37): Arg, Lys, His, or absent
XXXXXXSFSDXXXXXLDNLAXXDFXXWLIQTKXXXXX

SEQ ID NO: 4 - protein, 5 aa, Artificial Sequence
  Description of Artificial Sequence: Synthetic peptide
  MOD_RES (2)..(2): Met or an oxidatively stable Met replacement
EXNTI

SEQ ID NO: 5 - protein, 4 aa, Unknown
  Description of Unknown: GLP-2 analogue
YSKY

SEQ ID NO: 6 - protein, 37 aa, Artificial Sequence
  Description of Artificial Sequence: Synthetic polypeptide
  MOD_RES (1)..(1): Arg or absent
  MOD_RES (2)..(2): Arg or absent
  MOD_RES (15)..(15): Neutral/polar/large/nonaromatic residue such as Ile or Val
  MOD_RES (18)..(18): Neutral/polar residue such as Asn or Ser
  MOD_RES (21)..(21): Neutral residue such as Ala or Thr
  MOD_RES (29)..(29): Neutral/polar/large/nonaromatic residue such as Ile or Leu
  MOD_RES (30)..(30): Neutral or basic residue such as Gln or His
  MOD_RES (36)..(36): Arg, Lys, or absent
  MOD_RES (37)..(37): Lys or absent
XXHADGSFSDEMNTXLDXLAXRDFINWLXXTKITDXX

SEQ ID NO: 7 - protein, 37 aa, Artificial Sequence
  Description of Artificial Sequence: Synthetic polypeptide
  MOD_RES (1)..(1): Arg or absent
  MOD_RES (2)..(2): Arg or absent
  MOD_RES (21)..(21): Neutral residue such as Ala or Thr
  MOD_RES (36)..(36): Arg, Lys, or absent
  MOD_RES (37)..(37): Lys or absent
XXHADGSFSDEMNTILDNLAXRDFINWLIQTKITDXX

SEQ ID NO: 8 - protein, 33 aa, Unknown
  Description of Unknown: GLP-2 analogue
HADGSFSDEMNTILDNLATRDFINWLIQTKITD

SEQ ID NO: 9 - protein, 37 aa, Artificial Sequence
  Description of Artificial Sequence: Synthetic polypeptide
  MOD_RES (1)..(1): His, Arg, Lys, or absent
  MOD_RES (2)..(2): His, Arg, Lys, or absent
  MOD_RES (15)..(15): Met, Leu, Ile, Val, or Cys
  MOD_RES (18)..(18): Ala, Ser, Thr, Pro, Gly, Asn, Asp, Glu, or Gln
  MOD_RES (21)..(21): Ala, Ser, Thr, Pro, or Gly
  MOD_RES (22)..(22): His, Arg, or Lys
  MOD_RES (29)..(29): Met, Leu, Ile, Val, or Cys
  MOD_RES (30)..(30): Asn, Asp, Glu, Gln, His, Arg, or Lys
  MOD_RES (36)..(36): His, Arg, Lys, or absent
  MOD_RES (37)..(37): His, Arg, Lys, or absent
XXHADGSFSDEMNTXLDXLAXXDFINWLXXTKITDXX

SEQ ID NO: 10 - protein, 37 aa, Artificial Sequence; identical to SEQ ID NO: 7
  Description of Artificial Sequence: Synthetic polypeptide
  MOD_RES (1)..(1): His, Arg, Lys, or absent
  MOD_RES (2)..(2): His, Arg, Lys, or absent
  MOD_RES (21)..(21): Ala, Ser, Thr, Pro, or Gly
  MOD_RES (36)..(36): His, Arg, Lys, or absent
  MOD_RES (37)..(37): His, Arg, Lys, or absent

SEQ ID NO: 11 - protein, 39 aa, Artificial Sequence
  Description of Artificial Sequence: Synthetic polypeptide
  GLP-2 analogue
HGEGTFSDELATILDALAARDFIAWLIATKITDKKKKKK

SEQ ID NO: 12 - protein, 35 aa, Artificial Sequence
  Description of Artificial Sequence: Synthetic polypeptide
  GLP-2 analogue
HGEGTFSDELATILDALAARIFIAWLIATKKKKKK

SEQ ID NO: 13 - protein, 33 aa, Artificial Sequence
  Description of Artificial Sequence: Synthetic polypeptide
  GLP-2 analogue
HGDGSPSDELATILDALAARDFIAWLIATKITD

SEQ ID NO: 14 - protein, 33 aa, Artificial Sequence
  Description of Artificial Sequence: Synthetic polypeptide
  GLP-2 analogue
HGEGSFSDELATILDNLAARDFIAWLIQTKITD

SEQ ID NO: 15 - protein, 33 aa, Artificial Sequence
  Description of Artificial Sequence: Synthetic polypeptide
  GLP-2 analogue
HGDGSFSDELATILDALAARDFIAWLIATKITD

SEQ ID NO: 16 - protein, 33 aa, Artificial Sequence
  Description of Artificial Sequence: Synthetic polypeptide
  GLP-2 analogue
HGDGSFSDELATILDNLAARDFIAWLIATKITD

SEQ ID NO: 17 - protein, 33 aa, Artificial Sequence
  Description of Artificial Sequence: Synthetic polypeptide
  GLP-2 analogue
HGEGSFSDELATILDALAARDFIAWLIATKITD

SEQ ID NO: 18 - protein, 35 aa, Artificial Sequence
  Description of Artificial Sequence: Synthetic polypeptide
  GLP-2 analogue
HGDGSFSSELATILDNLAARDFIAWLIQTKKKKKK

SEQ ID NO: 19 - protein, 35 aa, Artificial Sequence
  Description of Artificial Sequence: Synthetic polypeptide
  GLP-2 analogue
HGDGSFSDELSTILDNLAARDFIAWLIQTKKKKKK

SEQ ID NO: 20 - protein, 35 aa, Artificial Sequence
  Description of Artificial Sequence: Synthetic polypeptide
  GLP-2 analogue
HGDGSFTSELATILDNLAARDFIAWLIQTKKKKKK

SEQ ID NO: 21 - protein, 35 aa, Artificial Sequence
  Description of Artificial Sequence: Synthetic polypeptide
  GLP-2 analogue
HGDGSFSDELKTILDNLAARDFIAWLIQTKKKKKK

SEQ ID NO: 22 - protein, 35 aa, Artificial Sequence
  Description of Artificial Sequence: Synthetic polypeptide
  GLP-2 analogue
HGDGSFTDELKTILDNLAARDFIAWLIQTKKKKKK

SEQ ID NO: 23 - protein, 35 aa, Artificial Sequence
  Description of Artificial Sequence: Synthetic polypeptide
  GLP-2 analogue
HGDGSFTSELKTILDNLAARDFIAWLIQTKKKKKK

SEQ ID NO: 24 - protein, 35 aa, Artificial Sequence
  Description of Artificial Sequence: Synthetic polypeptide
  GLP-2 analogue
HGDGSFTDELATILDNLAARDFIAWLIQTKKKKKK

SEQ ID NO: 25 - protein, 30 aa, Artificial Sequence
  Description of Artificial Sequence: Synthetic polypeptide
  GLP-2 analogue
HGDGSFSSELATILDNLAARDFIAWLIQTK

SEQ ID NO: 26 - protein, 39 aa, Artificial Sequence
  Description of Artificial Sequence: Synthetic polypeptide
  GLP-2 analogue
HGDGSFSDELNTILDNLAARDFIAWLIQTKITDKKKKKK

SEQ ID NO: 27 - protein, 35 aa, Artificial Sequence
  Description of Artificial Sequence: Synthetic polypeptide
  GLP-2 analogue
HGDGSFTDELSTILDNLAARDFIAWLIQTKKKKKK

SEQ ID NO: 28 - protein, 35 aa, Artificial Sequence
  Description of Artificial Sequence: Synthetic polypeptide
  GLP-2 analogue
HGDGSFTSELSTILDNLAARDFIAWLIQTKKKKKK

SEQ ID NO: 29 - protein, 35 aa, Artificial Sequence
  Description of Artificial Sequence: Synthetic polypeptide
  GLP-2 analogue
HGDGSFSSELSTILDNLAARDFIAWLIQTKKKKKK

SEQ ID NO: 30 - protein, 30 aa, Artificial Sequence
  Description of Artificial Sequence: Synthetic polypeptide
  GLP-2 analogue
HGDGSFSDELSTILDNLAARDFIAWLIQTK

SEQ ID NO: 31 - protein, 30 aa, Artificial Sequence
  Description of Artificial Sequence: Synthetic polypeptide
  GLP-2 analogue
HGDGSFTDELSTILDNLAARDFIAWLIQTK

SEQ ID NO: 32 - protein, 30 aa, Artificial Sequence
  Description of Artificial Sequence: Synthetic polypeptide
  GLP-2 analogue
HGDGSFTSELSTILDNLAARDFIAWLIQTK

SEQ ID NO: 33 - protein, 30 aa, Artificial Sequence
  Description of Artificial Sequence: Synthetic polypeptide
  GLP-2 analogue
HGDGSFSSELSTILDNLAARDFIAWLIQTK

SEQ ID NO: 34 - protein, 30 aa, Artificial Sequence
  Description of Artificial Sequence: Synthetic polypeptide
  GLP-2 analogue
HGDGSFTSELATILDNLAARDFIAWLIQTK

SEQ ID NO: 35 - protein, 30 aa, Artificial Sequence
  Description of Artificial Sequence: Synthetic polypeptide
  GLP-2 analogue
HGDGSFSDELKTILDNLAARDFIAWLIQTK

SEQ ID NO: 36 - protein, 30 aa, Artificial Sequence
  Description of Artificial Sequence: Synthetic polypeptide
  GLP-2 analogue
HGDGSFTDELKTILDNLAARDFIAWLIQTK

SEQ ID NO: 37 - protein, 39 aa, Artificial Sequence
  Description of Artificial Sequence: Synthetic polypeptide
  GLP-2 analogue
HGDGSFSDELATILDNLAARDFIAWLIQTKITDKKKKKK

SEQ ID NO: 38 - protein, 33 aa, Artificial Sequence
  Description of Artificial Sequence: Synthetic polypeptide
  GLP-2 analogue
HGDGSFSDELATILDNLAARDFIAWLIQTKITD

SEQ ID NO: 39 - protein, 30 aa, Artificial Sequence
  Description of Artificial Sequence: Synthetic polypeptide
  GLP-2 analogue
HGDGSFSDELATILDNLAARDFIAWLIQTK

SEQ ID NO: 40 - protein, 30 aa, Artificial Sequence
  Description of Artificial Sequence: Synthetic polypeptide
  GLP-2 analogue
HGDGSFTSELKTILDNLAARDFIAWLIQTK

SEQ ID NO: 41 - protein, 30 aa, Artificial Sequence
  Description of Artificial Sequence: Synthetic polypeptide
  GLP-2 analogue
HGDGSFTDELATILDNLAARDFIAWLIQTK

SEQ ID NO: 42 - protein, 39 aa, Artificial Sequence
  Description of Artificial Sequence: Synthetic polypeptide
  GLP-2 analogue
HGEGTFSSELSTILDALAARDFIAWLIATKITDKKKKKK

SEQ ID NO: 43 - protein, 39 aa, Artificial Sequence
  Description of Artificial Sequence: Synthetic polypeptide
  GLP-2 analogue
HGEGTFSDELSTILDALAARDFIAWLIATKITDKKKKKK

SEQ ID NO: 44 - protein, 39 aa, Artificial Sequence
  Description of Artificial Sequence: Synthetic polypeptide
  GLP-2 analogue
HGEGSFSSELSTILDALAARDFIAWLIATKITDKKKKKK

SEQ ID NO: 45 - protein, 39 aa, Artificial Sequence
  Description of Artificial Sequence: Synthetic polypeptide
  GLP-2 analogue
HGEGSFSDELSTILDALAARDFIAWLIATKITDKKKKKK

SEQ ID NO: 46 - protein, 39 aa, Artificial Sequence
  Description of Artificial Sequence: Synthetic polypeptide
  GLP-2 analogue
HGEGTFSSELATILDALAARDFIAWLIATKITDKKKKKK

SEQ ID NO: 47 - protein, 39 aa, Artificial Sequence
  Description of Artificial Sequence: Synthetic polypeptide
  GLP-2 analogue
HGEGSFSSELATILDALAARDFIAWLIATKITDKKKKKK

SEQ ID NO: 48 - protein, 39 aa, Artificial Sequence
  Description of Artificial Sequence: Synthetic polypeptide
  GLP-2 analogue
HGEGSFSDELKTILDALAARDFIAWLIATKITDKKKKKK

SEQ ID NO: 49 - protein, 39 aa, Artificial Sequence
  Description of Artificial Sequence: Synthetic polypeptide
  GLP-2 analogue
HGEGTFSDELKTILDALAARDFIAWLIATKITDKKKKKK

SEQ ID NO: 50 - protein, 39 aa, Artificial Sequence
  Description of Artificial Sequence: Synthetic polypeptide
  GLP-2 analogue
HGEGTFSSELKTILDALAARDFIAWLIATKITDKKKKKK

SEQ ID NO: 51 - protein, 33 aa, Artificial Sequence
  Description of Artificial Sequence: Synthetic polypeptide
  GLP-2 analogue
HGEGTFSSELSTILDALAARDFIAWLIATKITD

SEQ ID NO: 52 - protein, 33 aa, Artificial Sequence
  Description of Artificial Sequence: Synthetic polypeptide
  GLP-2 analogue
HGEGTFSDELSTILDALAARDFIAWLIATKITD

SEQ ID NO: 53 - protein, 33 aa, Artificial Sequence
  Description of Artificial Sequence: Synthetic polypeptide
  GLP-2 analogue
HGEGSFSSELSTILDALAARDFIAWLIATKITD

SEQ ID NO: 54 - protein, 33 aa, Artificial Sequence
  Description of Artificial Sequence: Synthetic polypeptide
  GLP-2 analogue
HGEGSFSDELSTILDALAARDFIAWLIATKITD

SEQ ID NO: 55 - protein, 33 aa, Artificial Sequence
  Description of Artificial Sequence: Synthetic polypeptide
  GLP-2 analogue
HGEGTFSSELATILDALAARDFIAWLIATKITD

SEQ ID NO: 56 - protein, 33 aa, Artificial Sequence
  Description of Artificial Sequence: Synthetic polypeptide
  GLP-2 analogue
HGEGSFSSELATILDALAARDFIAWLIATKITD

SEQ ID NO: 57 - protein, 33 aa, Artificial Sequence
  Description of Artificial Sequence: Synthetic polypeptide
  GLP-2 analogue
HGEGSFSDELKTILDALAARDFIAWLIATKITD

SEQ ID NO: 58 - protein, 33 aa, Artificial Sequence
  Description of Artificial Sequence: Synthetic polypeptide
  GLP-2 analogue
HGEGTFSDELKTILDALAARDFIAWLIATKITD

SEQ ID NO: 59 - protein, 33 aa, Artificial Sequence
  Description of Artificial Sequence: Synthetic polypeptide
  GLP-2 analogue
HGEGTFSSELKTILDALAARDFIAWLIATKITD

SEQ ID NO: 60 - protein, 73 aa, Artificial Sequence
  Description of Artificial Sequence: Synthetic polypeptide
  GLP-2 analogue
  MOD_RES (1)..(20): Ala, Leu, Ser, Thr, Tyr, Asn, Gln, Asp, Glu, Lys, Arg, His, Met, Orn, or absent
  MOD_RES (22)..(22): Gly, Ala or Sar
  MOD_RES (23)..(23): Glu or Asp
  MOD_RES (25)..(25): Ser or Thr
  MOD_RES (26)..(26): Phe or Pro
  MOD_RES (27)..(27): Ser or Thr
  MOD_RES (28)..(28): Asp or Ser
  MOD_RES (29)..(29): Glu or Asp
  MOD_RES (30)..(30): Met, Leu, Nle, or an oxidatively stable Met-replacement amino acid
  MOD_RES (31)..(31): Asn, Ala, Lys, or Ser
  MOD_RES (32)..(32): Thr or Lys
  MOD_RES (33)..(33): Ile, Glu or Gln
  MOD_RES (34)..(34): Leu, Met, or Nle
  MOD_RES (35)..(35): Asp or Glu
  MOD_RES (36)..(36): Asn or Ala
  MOD_RES (37)..(37): Leu or Glu
  MOD_RES (38)..(38): Ala or Aib
  MOD_RES (39)..(39): Ala or Thr
  MOD_RES (40)..(40): Arg or Lys
  MOD_RES (41)..(41): Asp or Ile
  MOD_RES (44)..(44): Asn, Ala, or Glu
  MOD_RES (48)..(48): Gln, Ala, or Asn
  MOD_RES (51)..(51): Pro Ile, or absent
  MOD_RES (52)..(52): Thr or absent
  MOD_RES (53)..(53): Asp, Asn, or absent
  MOD_RES (54)..(73): Ala, Leu, Ser, Thr, Tyr, Asn, Gln, Asp, Glu, Lys, Arg, His, Met, Orn, or absent
XXXXXXXXXXXXXXXXXXXXHXXGXXXXXXXXXXXXXXXXXFIXWLIXTKXXXXXXXXXXXXXXXXXXXXXXX

SEQ ID NO: 61 - protein, 73 aa, Artificial Sequence
  Description of Artificial Sequence: Synthetic polypeptide
  GLP-2 analogue
  MOD_RES (1)..(20): Ala, Leu, Ser, Thr, Tyr, Asn, Gln, Asp, Glu, Lys, Arg, His, Met, Orn, or absent
  MOD_RES (23)..(23): Glu or Asp
  MOD_RES (25)..(25): Ser or Thr
  MOD_RES (27)..(27): Ser or Thr
  MOD_RES (28)..(28): Asp or Ser
  MOD_RES (29)..(29): Glu or Asp
  MOD_RES (30)..(30): Met, Leu, Nle, or an oxidatively stable Met-replacement amino acid
  MOD_RES (31)..(31): Asn, Ala, Lys or Ser
  MOD_RES (32)..(32): Thr or Lys
  MOD_RES (33)..(33): Ile, Glu, or Gln
  MOD_RES (34)..(34): Leu, Met or Nle
  MOD_RES (35)..(35): Asp or Glu
  MOD_RES (36)..(36): Asn or Ala
  MOD_RES (37)..(37): Leu or Glu
  MOD_RES (39)..(39): Ala or Thr
  MOD_RES (44)..(44): Asn or Ala
  MOD_RES (48)..(48): Gln, Ala, or Asn
  MOD_RES (51)..(51): Pro, Ile, or absent
  MOD_RES (52)..(52): Thr or absent
  MOD_RES (53)..(53): Asp or absent
  MOD_RES (54)..(73): Ala, Leu, Ser, Thr, Tyr, Asn, Gln, Asp, Glu, Lys, Arg, His, Met, Orn, or absent
XXXXXXXXXXXXXXXXXXXXHGXGXFXXXXXXXXXXXAXRDFIXWLIXTKXXXXXXXXXXXXXXXXXXXXXXX

SEQ ID NO: 62 - protein, 73 aa, Artificial Sequence
  Description of Artificial Sequence: Synthetic polypeptide
  GLP-2 analogue
  MOD_RES (1)..(20): Ala, Leu, Ser, Thr, Tyr, Asn, Gln,  Asp, Glu, Lys, Arg, His, Met, Orn, or absent
  MOD_RES (23)..(23): Glu or Asp
  MOD_RES (25)..(25): Ser or Thr
  MOD_RES (27)..(27): Ser or Thr
  MOD_RES (28)..(28): Asp or Ser
  MOD_RES (30)..(30): Met, Leu, Nle, or an oxidatively stable Met-replacement amino acid
  MOD_RES (31)..(31): Asn, Ala, Lys, or Ser
  MOD_RES (36)..(36): Asn or Ala
  MOD_RES (44)..(44): Asn or Ala
  MOD_RES (48)..(48): Gln or Ala
  MOD_RES (51)..(51): Pro or absent
  MOD_RES (52)..(52): Thr or absent
  MOD_RES (53)..(53): Asp or absent
  MOD_RES (54)..(73): Ala, Leu, Ser, Thr, Tyr, Asn, Gln, Asp, Glu, Lys, Arg, His, Met, Orn, or absent
XXXXXXXXXXXXXXXXXXXXHGXGXFXXEXXTILDXLAARDFIXWLIXTKXXXXXXXXXXXXXXXXXXXXXXX

SEQ ID NO: 63 - protein, 34 aa, Homo sapiens
HADGSFSDEMNTILDNLAARDFINWLIQTKITDR